European Patent Specification EP 4 188 457 B1, published July 3, 2024. Title: CONJUGATE OR ITS SALT COMPRISING A GASTRIN-RELEASING PEPTIDE RECEPTOR ANTAGONIST AND USES THEREOF. Applicant: Orano Med. Application PCT/EPXX/XXXXX. The sequence listing filed with the application follows.

SEQUENCE LISTING (2 sequences)

SEQ ID NO: 1 - protein, 9 aa, Artificial Sequence
  Gastrin-releasing peptide receptor (GRPR) antagonist  peptide known as JMV 594
  MISC_FEATURE (1)..(1): D-Phe
  MISC_FEATURE (8)..(8): Statine
  MISC_FEATURE (9)..(9): Leu-NH2
FQYAVGHXL

SEQ ID NO: 2 - protein, 11 aa, Artificial Sequence
  Synthetic peptide
  MISC_FEATURE (1)..(1): Beta-Ala
  MISC_FEATURE (2)..(2): Beta-Ala
  MISC_FEATURE (3)..(3): D-Phe
  MISC_FEATURE (10)..(10): Statine
  MISC_FEATURE (11)..(11): Leu-NH2
AAFQYAVGHXL